European Patent Specification EP 3 833 743 B1, published January 24, 2024. Title: RECOMBINANT CD1-RESTRICTED T CELLS AND METHODS. Applicant: NantBio. The sequence listing filed with the application follows.

SEQUENCE LISTING (4 sequences)

SEQ ID NO: 1 - DNA, 807 bp, Homo sapiens
  misc_feature (1)..(807): TCR 18 alpha
atgtggggagttttccttctttatgtttccatgaagatgggaggcactacaggacaaaacattgaccagcccactgagatgacagctacggaaggtgccattgtccagatcaactgcacgtaccagacatctgggttcaacgggctgttctggtaccagcaacatgctggcgaagcacccacatttctgtcttacaatgttctggatggtttggaggagaaaggtcgtttttcttcattccttagtcggtctaaagggtacagttacctccttttgaaggagctccagatgaaagactctgcctcttacctctgtgctgtcctaaatactggaggcttcaaaactatctttggagcaggaacaagactatttgttaaagcaaatatccagaaccctgaccctgccgtgtaccagctgagagactctaaatccagtgacaagtctgtctgcctattcaccgattttgattctcaaacaaatgtgtcacaaagtaaggattctgatgtgtatatcacagacaaaactgtgctagacatgaggtctatggacttcaagagcaacagtgctgtggcctggagcaacaaatctgactttgcatgtgcaaacgccttcaacaacagcattattccagaagacaccttcttccccagcccagaaagttcctgtgatgtcaagctggtcgagaaaagctttgaaacagatacgaacctaaactttcaaaacctgtcagtgattgggttccgaatcctcctcctgaaagtggccgggtttaatctgctcatgacgctgcggctgtggtccagctga

SEQ ID NO: 2 - protein, 268 aa, Homo sapiens [sequence omitted]

SEQ ID NO: 3 - DNA, 954 bp, Homo sapiens
  misc_feature (1)..(954): TCR 18 beta
atgagcctcgggctcctgtgctgtggggccttttctctcctgtgggcaggtccagtgaatgctggtgtcactcagaccccaaaattccgggtcctgaagacaggacagagcatgacactgctgtgtgcccaggatatgaaccatgaatacatgtactggtatcgacaagacccaggcatggggctgaggctgattcattactcagttggtgagggtacaactgccaaaggagaggtccctgatggctacaatgtctccagattaaaaaaacagaatttcctgctggggttggagtcggctgctccctcccaaacatctgtgtacttctgtgccagcagaccccccttgacagctaggggccttaaacacaccggggagctgttttttggagaaggctctaggctgaccgtactggaggacctgaaaaacgtgttcccacccgaggtcgctgtgtttgagccatcagaagcagagatctcccacacccaaaaggccacactggtgtgcctggccacaggcttctaccccgaccacgtggagctgagctggtgggtgaatgggaaggaggtgcacagtggggtcagcacagacccgcagcccctcaaggagcagcccgccctcaatgactccagatactgcctgagcagccgcctgagggtctcggccaccttctggcagaacccccgcaaccacttccgctgtcaagtccagttctacgggctctcggagaatgacgagtggacccaggatagggccaaacctgtcacccagatcgtcagcgccgaggcctggggtagagcagactgtggcttcacctccgagtcttaccagcaaggggtcctgtctgccaccatcctctatgagatcttgctagggaaggccaccttgtatgccgtgctggtcagtgccctcgtgctgatggccatggtcaagagaaaggattccagaggctag

SEQ ID NO: 4 - protein, 317 aa, Homo sapiens [sequence omitted]